European Patent Specification EP 3 717 644 B1, published September 30, 2026. Title: DETECTING BREAST CANCER. Applicant: MAYO FOUNDATION FOR MEDICAL EDUCATION AND RESEARCH EXACT SCIENCES DEVELOPMENT COMPANY, LLC. Application PCT/US2018/062809. The sequence listing filed with the application follows.

SEQUENCE LISTING (464 sequences)

SEQ ID NO: 1 - DNA, 21 bp, Artificial Sequence
  Synthetic
gagtttcggcggcgtttttcg

SEQ ID NO: 2 - DNA, 22 bp, Artificial Sequence
  Synthetic
cgctacgtctaacttcccgcgc

SEQ ID NO: 3 - DNA, 29 bp, Artificial Sequence
  Synthetic
ttttcgacgagtaggattgaagaaggaac

SEQ ID NO: 4 - DNA, 25 bp, Artificial Sequence
  Synthetic
gcgaatctatctaccgaaacgcgct

SEQ ID NO: 5 - DNA, 31 bp, Artificial Sequence
  Synthetic
ttttgatttgtaatatagaggaaagcgtcgt

SEQ ID NO: 6 - DNA, 31 bp, Artificial Sequence
  Synthetic
gtataaacgcgtaaataccaaactaaacgaa

SEQ ID NO: 7 - DNA, 25 bp, Artificial Sequence
  Synthetic
gtttcgagaaaggagaagggggagc

SEQ ID NO: 8 - DNA, 25 bp, Artificial Sequence
  Synthetic
actcccaacgaaaacttcgcaaacg

SEQ ID NO: 9 - DNA, 23 bp, Artificial Sequence
  Synthetic
gttttttgtcgggagttattcgt

SEQ ID NO: 10 - DNA, 28 bp, Artificial Sequence
  Synthetic
ccaaaaattaaattaaaaacgctacgca

SEQ ID NO: 11 - DNA, 20 bp, Artificial Sequence
  Synthetic
gttttaggagggtggggcgt

SEQ ID NO: 12 - DNA, 25 bp, Artificial Sequence
  Synthetic
aacacgactattcgaaaaacgcgca

SEQ ID NO: 13 - DNA, 20 bp, Artificial Sequence
  Synthetic
ttcgtagtatcgggagtcga

SEQ ID NO: 14 - DNA, 24 bp, Artificial Sequence
  Synthetic
gaaataataaaaacgccgcacgct

SEQ ID NO: 15 - DNA, 25 bp, Artificial Sequence
  Synthetic
gtcgtagttttcgcgggtggtaagc

SEQ ID NO: 16 - DNA, 25 bp, Artificial Sequence
  Synthetic
cgaacgctacctaaactctcccgac

SEQ ID NO: 17 - DNA, 25 bp, Artificial Sequence
  Synthetic
ggaatcgcgagttttgggatagtcg

SEQ ID NO: 18 - DNA, 25 bp, Artificial Sequence
  Synthetic
aaatacaattacaccctctaccgcc

SEQ ID NO: 19 - DNA, 20 bp, Artificial Sequence
  Synthetic
gaggcgttcggtgggatttc

SEQ ID NO: 20 - DNA, 25 bp, Artificial Sequence
  Synthetic
ccccgacctataaacctacgacgct

SEQ ID NO: 21 - DNA, 20 bp, Artificial Sequence
  Synthetic
gaggaggtagcgggcgtcga

SEQ ID NO: 22 - DNA, 25 bp, Artificial Sequence
  Synthetic
cgcgtcgatctaacttacctacgaa

SEQ ID NO: 23 - DNA, 25 bp, Artificial Sequence
  Synthetic
ttgcgtttatcgatttcgttttcgt

SEQ ID NO: 24 - DNA, 29 bp, Artificial Sequence
  Synthetic
gcactactatcccccgaactactctacgc

SEQ ID NO: 25 - DNA, 24 bp, Artificial Sequence
  Synthetic
ttattaggcggggagtcgggtgtc

SEQ ID NO: 26 - DNA, 25 bp, Artificial Sequence
  Synthetic
ctcgaatccctaaaaaactcgcgaa

SEQ ID NO: 27 - DNA, 25 bp, Artificial Sequence
  Synthetic
aggaaattcggtagcgattatacgg

SEQ ID NO: 28 - DNA, 28 bp, Artificial Sequence
  Synthetic
aaacccctacaacctcaccgtacacgat

SEQ ID NO: 29 - DNA, 25 bp, Artificial Sequence
  Synthetic
cggagttaataggtacgggaggcgt

SEQ ID NO: 30 - DNA, 22 bp, Artificial Sequence
  Synthetic
caaacccccgaactatcgcgaa

SEQ ID NO: 31 - DNA, 22 bp, Artificial Sequence
  Synthetic
cgggtatcgcggttaagttggc

SEQ ID NO: 32 - DNA, 25 bp, Artificial Sequence
  Synthetic
tatcgtaaaaacccaacccctcgac

SEQ ID NO: 33 - DNA, 23 bp, Artificial Sequence
  Synthetic
gggattggtgagattcgggacgt

SEQ ID NO: 34 - DNA, 25 bp, Artificial Sequence
  Synthetic
ctccccgaaaccaaaaaacaacgaa

SEQ ID NO: 35 - DNA, 25 bp, Artificial Sequence
  Synthetic
gttttaaatcgtattcgtagttcgg

SEQ ID NO: 36 - DNA, 25 bp, Artificial Sequence
  Synthetic
acgaacgaaaactttcctaaacgaa

SEQ ID NO: 37 - DNA, 25 bp, Artificial Sequence
  Synthetic
gcgtttttttatcgttttagggcgt

SEQ ID NO: 38 - DNA, 24 bp, Artificial Sequence
  Synthetic
accgacactaccaacctctccgaa

SEQ ID NO: 39 - DNA, 22 bp, Artificial Sequence
  Synthetic
tgcggggatttttagcggaagc

SEQ ID NO: 40 - DNA, 28 bp, Artificial Sequence
  Synthetic
ccgacgaactatccgactatcactcgtt

SEQ ID NO: 41 - DNA, 24 bp, Artificial Sequence
  Synthetic
gtagtaggtggagggggcgagttc

SEQ ID NO: 42 - DNA, 24 bp, Artificial Sequence
  Synthetic
ctctcgaaaaccgcaaaatcctcg

SEQ ID NO: 43 - DNA, 27 bp, Artificial Sequence
  Synthetic
ggtaatattgcgatatttcgtagacgt

SEQ ID NO: 44 - DNA, 25 bp, Artificial Sequence
  Synthetic
aacaatcaaataatcgaacgcacgc

SEQ ID NO: 45 - DNA, 23 bp, Artificial Sequence
  Synthetic
gtcgtttttcgttacgaagcggc

SEQ ID NO: 46 - DNA, 25 bp, Artificial Sequence
  Synthetic
aaaactaaataaatctatcctcgat

SEQ ID NO: 47 - DNA, 24 bp, Artificial Sequence
  Synthetic
gcgtcggcggtttttagtaaaagc

SEQ ID NO: 48 - DNA, 25 bp, Artificial Sequence
  Synthetic
aacgaatctcattaaatctcccgtc

SEQ ID NO: 49 - DNA, 18 bp, Artificial Sequence
  Synthetic
gattttcgggagcggcga

SEQ ID NO: 50 - DNA, 18 bp, Artificial Sequence
  Synthetic
cttccccgcaacgaaccg

SEQ ID NO: 51 - DNA, 25 bp, Artificial Sequence
  Synthetic
ttcgttggtatattcgcgtaggtgc

SEQ ID NO: 52 - DNA, 26 bp, Artificial Sequence
  Synthetic
cgaataccgaaatctataaccccgaa

SEQ ID NO: 53 - DNA, 23 bp, Artificial Sequence
  Synthetic
attatgattacgatggttgacgg

SEQ ID NO: 54 - DNA, 25 bp, Artificial Sequence
  Synthetic
ctccataaaaacgaatttaaacgaa

SEQ ID NO: 55 - DNA, 25 bp, Artificial Sequence
  Synthetic
tttggttatagaacgtagaggtcgt

SEQ ID NO: 56 - DNA, 22 bp, Artificial Sequence
  Synthetic
atcgaaccaccaaaccaaacgc

SEQ ID NO: 57 - DNA, 22 bp, Artificial Sequence
  Synthetic
gggaagtttagtaggtgagcgt

SEQ ID NO: 58 - DNA, 25 bp, Artificial Sequence
  Synthetic
actaaaaacgtttccgtcgaacgca

SEQ ID NO: 59 - DNA, 25 bp, Artificial Sequence
  Synthetic
gttggtaggagtagggttggttcga

SEQ ID NO: 60 - DNA, 24 bp, Artificial Sequence
  Synthetic
atcgcaatcgtaacccgtaaacgc

SEQ ID NO: 61 - DNA, 25 bp, Artificial Sequence
  Synthetic
attcgtacggttttttcgttttcgt

SEQ ID NO: 62 - DNA, 23 bp, Artificial Sequence
  Synthetic
gaccaactacttccgctcgacgc

SEQ ID NO: 63 - DNA, 20 bp, Artificial Sequence
  Synthetic
cggatttagcggtcgagacg

SEQ ID NO: 64 - DNA, 23 bp, Artificial Sequence
  Synthetic
tttaaaacgtttctcgcgacgcc

SEQ ID NO: 65 - DNA, 24 bp, Artificial Sequence
  Synthetic
tcgttaggcgatgataattagcga

SEQ ID NO: 66 - DNA, 25 bp, Artificial Sequence
  Synthetic
taaaaaaaccataaaccctaacgac

SEQ ID NO: 67 - DNA, 25 bp, Artificial Sequence
  Synthetic
gttggagaagacgattcgttcggac

SEQ ID NO: 68 - DNA, 23 bp, Artificial Sequence
  Synthetic
ccaaaacctcactcctcaaccgc

SEQ ID NO: 69 - DNA, 19 bp, Artificial Sequence
  Synthetic
cgcgatgcgcgttttgaac

SEQ ID NO: 70 - DNA, 27 bp, Artificial Sequence
  Synthetic
gacgcgactaacttccaacctaacgaa

SEQ ID NO: 71 - DNA, 22 bp, Artificial Sequence
  Synthetic
ttttcgtggttgtcgtcgttgc

SEQ ID NO: 72 - DNA, 27 bp, Artificial Sequence
  Synthetic
gccgcgctctacactaaacatattcgc

SEQ ID NO: 73 - DNA, 23 bp, Artificial Sequence
  Synthetic
cggggaagtgggagtttttagcg

SEQ ID NO: 74 - DNA, 25 bp, Artificial Sequence
  Synthetic
aaaaaaactaaatcaaaaccgcgac

SEQ ID NO: 75 - DNA, 24 bp, Artificial Sequence
  Synthetic
gcgagttcgcgttgtttacgtttc

SEQ ID NO: 76 - DNA, 26 bp, Artificial Sequence
  Synthetic
accgacgctacctataactccacgct

SEQ ID NO: 77 - DNA, 25 bp, Artificial Sequence
  Synthetic
ttaggtttgtttattaattttacgt

SEQ ID NO: 78 - DNA, 18 bp, Artificial Sequence
  Synthetic
tctacaaaacgccgcgac

SEQ ID NO: 79 - DNA, 23 bp, Artificial Sequence
  Synthetic
gttaattcgagagcgcgaggcgt

SEQ ID NO: 80 - DNA, 28 bp, Artificial Sequence
  Synthetic
gaccaaaaaaaataaaaaatcccgcgac

SEQ ID NO: 81 - DNA, 27 bp, Artificial Sequence
  Synthetic
taaagaaatagaaagcgggcgatacgt

SEQ ID NO: 82 - DNA, 24 bp, Artificial Sequence
  Synthetic
cgaactaaaaaaaccgccaacccg

SEQ ID NO: 83 - DNA, 20 bp, Artificial Sequence
  Synthetic
gggttttgcggttaatggcg

SEQ ID NO: 84 - DNA, 25 bp, Artificial Sequence
  Synthetic
aataacaaacgcgtcccgaaaacga

SEQ ID NO: 85 - DNA, 32 bp, Artificial Sequence
  Synthetic
ttagttttttttggtttttatttgaatttcga

SEQ ID NO: 86 - DNA, 26 bp, Artificial Sequence
  Synthetic
aacttttccaccgattctcaattccg

SEQ ID NO: 87 - DNA, 25 bp, Artificial Sequence
  Synthetic
atttaaattttcggcgtttcgtcgt

SEQ ID NO: 88 - DNA, 27 bp, Artificial Sequence
  Synthetic
acactccaaatcgacctttacaatcgc

SEQ ID NO: 89 - DNA, 25 bp, Artificial Sequence
  Synthetic
agtttggttcgtttagcgattgcgt

SEQ ID NO: 90 - DNA, 25 bp, Artificial Sequence
  Synthetic
aacgcgactaaaaccaatttccgca

SEQ ID NO: 91 - DNA, 25 bp, Artificial Sequence
  Synthetic
tttatttgtttttatcgttcgtcgg

SEQ ID NO: 92 - DNA, 24 bp, Artificial Sequence
  Synthetic
aaatatatacccgatttccccgtt

SEQ ID NO: 93 - DNA, 25 bp, Artificial Sequence
  Synthetic
taatcggcgtcgagagagatatcgt

SEQ ID NO: 94 - DNA, 22 bp, Artificial Sequence
  Synthetic
ccgtcaaccaatcgaaaacgaa

SEQ ID NO: 95 - DNA, 25 bp, Artificial Sequence
  Synthetic
tcgtttatttcgttttttttgtcga

SEQ ID NO: 96 - DNA, 25 bp, Artificial Sequence
  Synthetic
aaccaacctaaaatctacactcgca

SEQ ID NO: 97 - DNA, 20 bp, Artificial Sequence
  Synthetic
gggtcgtaggggtttatcgc

SEQ ID NO: 98 - DNA, 26 bp, Artificial Sequence
  Synthetic
catacttatccgaacgtctaaacgtc

SEQ ID NO: 99 - DNA, 23 bp, Artificial Sequence
  Synthetic
ggttttagcgatgaatcggacgt

SEQ ID NO: 100 - DNA, 25 bp, Artificial Sequence
  Synthetic
cacgatcttaaaaaaacaacgcgac

SEQ ID NO: 101 - DNA, 25 bp, Artificial Sequence
  Synthetic
cgtatttttaggtttagttcggcgt

SEQ ID NO: 102 - DNA, 25 bp, Artificial Sequence
  Synthetic
acactattacccgcgaaaaaacgat

SEQ ID NO: 103 - DNA, 27 bp, Artificial Sequence
  Synthetic
gagtttgtttgggggttggtcgtattc

SEQ ID NO: 104 - DNA, 31 bp, Artificial Sequence
  Synthetic
ccaaatataacgtttaactctttaccacgaa

SEQ ID NO: 105 - DNA, 25 bp, Artificial Sequence
  Synthetic
ttttttttgattcggattttttcgg

SEQ ID NO: 106 - DNA, 25 bp, Artificial Sequence
  Synthetic
ctaataaacgccgccgtattcgacg

SEQ ID NO: 107 - DNA, 25 bp, Artificial Sequence
  Synthetic
ttttcgcgttgtttttatttatcgt

SEQ ID NO: 108 - DNA, 25 bp, Artificial Sequence
  Synthetic
tacacaaccacccaactactccgcg

SEQ ID NO: 109 - DNA, 25 bp, Artificial Sequence
  Synthetic
tgttgttgggtaaaggttagtacgt

SEQ ID NO: 110 - DNA, 19 bp, Artificial Sequence
  Synthetic
cgaaaacccaactcccgaa

SEQ ID NO: 111 - DNA, 23 bp, Artificial Sequence
  Synthetic
tttttgcggtcgtttttcggagc

SEQ ID NO: 112 - DNA, 25 bp, Artificial Sequence
  Synthetic
cttaccaactaacccccgcctaccg

SEQ ID NO: 113 - DNA, 24 bp, Artificial Sequence
  Synthetic
cgttttagtagggattgggggcga

SEQ ID NO: 114 - DNA, 25 bp, Artificial Sequence
  Synthetic
cccgaaaaccaaaataaaatccgca

SEQ ID NO: 115 - DNA, 23 bp, Artificial Sequence
  Synthetic
cggaatagcgcggtcgttttttc

SEQ ID NO: 116 - DNA, 24 bp, Artificial Sequence
  Synthetic
tttaaccgtaacgctcgcctcgac

SEQ ID NO: 117 - DNA, 25 bp, Artificial Sequence
  Synthetic
gtcggttgtgtttagagcgtagcgt

SEQ ID NO: 118 - DNA, 21 bp, Artificial Sequence
  Synthetic
aaaaaaaaccccgacgacgaa

SEQ ID NO: 119 - DNA, 24 bp, Artificial Sequence
  Synthetic
gttgcgattgtttgtattttgcgg

SEQ ID NO: 120 - DNA, 25 bp, Artificial Sequence
  Synthetic
ataataacaaaaaacccctcccgac

SEQ ID NO: 121 - DNA, 25 bp, Artificial Sequence
  Synthetic
agtttcgttagggaagggttgcgtc

SEQ ID NO: 122 - DNA, 25 bp, Artificial Sequence
  Synthetic
caactaaaactctaccgcgctcgat

SEQ ID NO: 123 - DNA, 25 bp, Artificial Sequence
  Synthetic
aggaagggtttcgagtttagtgcgg

SEQ ID NO: 124 - DNA, 25 bp, Artificial Sequence
  Synthetic
aaaaaaatcaacgcgtcctcctcgc

SEQ ID NO: 125 - DNA, 25 bp, Artificial Sequence
  Synthetic
tttcgatttcgtttttaaatttcgt

SEQ ID NO: 126 - DNA, 25 bp, Artificial Sequence
  Synthetic
aaactaaacgacctaaccctacgta

SEQ ID NO: 127 - DNA, 25 bp, Artificial Sequence
  Synthetic
aagtttacgcgcgagtttgatcgtc

SEQ ID NO: 128 - DNA, 22 bp, Artificial Sequence
  Synthetic
cgaaacgacttctctccccgca

SEQ ID NO: 129 - DNA, 25 bp, Artificial Sequence
  Synthetic
tttagttcgcggaagttaggttcgg

SEQ ID NO: 130 - DNA, 24 bp, Artificial Sequence
  Synthetic
gaaaacacaataaaccccgccgtc

SEQ ID NO: 131 - DNA, 25 bp, Artificial Sequence
  Synthetic
gttagattgtaggagggattagcgg

SEQ ID NO: 132 - DNA, 25 bp, Artificial Sequence
  Synthetic
aaaaaacgactaaaaaattcacgcc

SEQ ID NO: 133 - DNA, 25 bp, Artificial Sequence
  Synthetic
tttggagtttgggggatcgatagtc

SEQ ID NO: 134 - DNA, 25 bp, Artificial Sequence
  Synthetic
cgacgaaactaaaaccgcgtacgta

SEQ ID NO: 135 - DNA, 25 bp, Artificial Sequence
  Synthetic
tttggagtttgggggatcgatagtc

SEQ ID NO: 136 - DNA, 25 bp, Artificial Sequence
  Synthetic
cgacgaaactaaaaccgcgtacgta

SEQ ID NO: 137 - DNA, 25 bp, Artificial Sequence
  Synthetic
attatattgggggcgttaggttcgg

SEQ ID NO: 138 - DNA, 25 bp, Artificial Sequence
  Synthetic
aacaaacaattcgcacgtaaacgaa

SEQ ID NO: 139 - DNA, 31 bp, Artificial Sequence
  Synthetic
gggcggtttacgtggatttttatagattttc

SEQ ID NO: 140 - DNA, 25 bp, Artificial Sequence
  Synthetic
gcgtctcgaaccgtaccctaacgta

SEQ ID NO: 141 - DNA, 24 bp, Artificial Sequence
  Synthetic
cgtcgttgttgattatgatcgcgg

SEQ ID NO: 142 - DNA, 24 bp, Artificial Sequence
  Synthetic
cgcttcctaacaaccttcctcgaa

SEQ ID NO: 143 - DNA, 25 bp, Artificial Sequence
  Synthetic
ttaacggtattttttgttttttcgt

SEQ ID NO: 144 - DNA, 22 bp, Artificial Sequence
  Synthetic
aaaaaaaactcgtccccgcgct

SEQ ID NO: 145 - DNA, 28 bp, Artificial Sequence
  Synthetic
tcggttagttcgaggtaggaagttttgc

SEQ ID NO: 146 - DNA, 30 bp, Artificial Sequence
  Synthetic
tattaaccgaaaaacgaaaaccaaatccga

SEQ ID NO: 147 - DNA, 25 bp, Artificial Sequence
  Synthetic
agttttgttgttttgggtaggtcgg

SEQ ID NO: 148 - DNA, 25 bp, Artificial Sequence
  Synthetic
aaaaactaaaaacctttctctcgac

SEQ ID NO: 149 - DNA, 28 bp, Artificial Sequence
  Synthetic
gcgttgagagtgacggatatttttcgtc

SEQ ID NO: 150 - DNA, 25 bp, Artificial Sequence
  Synthetic
actacctaaactccgaacacgcccg

SEQ ID NO: 151 - DNA, 25 bp, Artificial Sequence
  Synthetic
ttagcgtatcgggaattagggggac

SEQ ID NO: 152 - DNA, 22 bp, Artificial Sequence
  Synthetic
gaaaacgaaaaaacgacgcgca

SEQ ID NO: 153 - DNA, 25 bp, Artificial Sequence
  Synthetic
tcgttttttaggtggggaagaagcg

SEQ ID NO: 154 - DNA, 26 bp, Artificial Sequence
  Synthetic
gaaccgtatttaaaaccaatccccgc

SEQ ID NO: 155 - DNA, 23 bp, Artificial Sequence
  Synthetic
aattggggttcggggttcggtac

SEQ ID NO: 156 - DNA, 25 bp, Artificial Sequence
  Synthetic
ttacccctacccaaaaaaatacgct

SEQ ID NO: 157 - DNA, 22 bp, Artificial Sequence
  Synthetic
ggggttagagtttcgcgttcgc

SEQ ID NO: 158 - DNA, 28 bp, Artificial Sequence
  Synthetic
cgcgtctcccgtcctatctatatacgtc

SEQ ID NO: 159 - DNA, 27 bp, Artificial Sequence
  Synthetic
taggaattttttaaattcgttttacgg

SEQ ID NO: 160 - DNA, 26 bp, Artificial Sequence
  Synthetic
cacaaaaactcgatacaattaccgtt

SEQ ID NO: 161 - DNA, 25 bp, Artificial Sequence
  Synthetic
tattttatagtcgcgttaaaagcgt

SEQ ID NO: 162 - DNA, 25 bp, Artificial Sequence
  Synthetic
gtcgataaaaaacctacgcgacgaa

SEQ ID NO: 163 - DNA, 26 bp, Artificial Sequence
  Synthetic
gatttagtttttcgggtttatagcgg

SEQ ID NO: 164 - DNA, 25 bp, Artificial Sequence
  Synthetic
tattaaaaacgaccaaacctccgca

SEQ ID NO: 165 - DNA, 26 bp, Artificial Sequence
  Synthetic
tggttgtaggcgttttgttggagttc

SEQ ID NO: 166 - DNA, 25 bp, Artificial Sequence
  Synthetic
aaaaacgaccctaaccaccctcgtt

SEQ ID NO: 167 - DNA, 25 bp, Artificial Sequence
  Synthetic
ttttgcgtagttgggtagggttcgg

SEQ ID NO: 168 - DNA, 23 bp, Artificial Sequence
  Synthetic
cccgcattcccgaaaaaaacgat

SEQ ID NO: 169 - DNA, 25 bp, Artificial Sequence
  Synthetic
ttagggtttttttcgaggagttcga

SEQ ID NO: 170 - DNA, 24 bp, Artificial Sequence
  Synthetic
atcccccgtacgaaactaaacgcg

SEQ ID NO: 171 - DNA, 23 bp, Artificial Sequence
  Synthetic
gcgttcgtattttcgggagaggc

SEQ ID NO: 172 - DNA, 25 bp, Artificial Sequence
  Synthetic
tctacgtaactaaacaaaacccgaa

SEQ ID NO: 173 - DNA, 33 bp, Artificial Sequence
  Synthetic
cgttttgtgttttataaaaagaaagattttcgg

SEQ ID NO: 174 - DNA, 21 bp, Artificial Sequence
  Synthetic
aaaaccccaaaaacgcccgat

SEQ ID NO: 175 - DNA, 27 bp, Artificial Sequence
  Synthetic
ggggcgtatatattagttatcgagcga

SEQ ID NO: 176 - DNA, 25 bp, Artificial Sequence
  Synthetic
aaaaaaaaccctaaaaaccgccgaa

SEQ ID NO: 177 - DNA, 26 bp, Artificial Sequence
  Synthetic
ttcgtttaatgagaaggggttagcgg

SEQ ID NO: 178 - DNA, 31 bp, Artificial Sequence
  Synthetic
taaaacaaactaaaaaccttaacgcgacgct

SEQ ID NO: 179 - DNA, 20 bp, Artificial Sequence
  Synthetic
ggggagggagttttttttac

SEQ ID NO: 180 - DNA, 25 bp, Artificial Sequence
  Synthetic
gtacgcgaactcgccaaacactacg

SEQ ID NO: 181 - DNA, 25 bp, Artificial Sequence
  Synthetic
gtagggttggtagtcgtttttacgt

SEQ ID NO: 182 - DNA, 28 bp, Artificial Sequence
  Synthetic
aacccatctaattacaaaatacctcgat

SEQ ID NO: 183 - DNA, 26 bp, Artificial Sequence
  Synthetic
ggttttataggggaaattattttcgt

SEQ ID NO: 184 - DNA, 25 bp, Artificial Sequence
  Synthetic
aaaacctcgtctttataacatcgaa

SEQ ID NO: 185 - DNA, 27 bp, Artificial Sequence
  Synthetic
taggatatttcgatgttataaagacga

SEQ ID NO: 186 - DNA, 25 bp, Artificial Sequence
  Synthetic
aacaaaactaacaaccgcctccacg

SEQ ID NO: 187 - DNA, 27 bp, Artificial Sequence
  Synthetic
tttggagttatcggaaggcgaaagtac

SEQ ID NO: 188 - DNA, 24 bp, Artificial Sequence
  Synthetic
gcacgccgaaaaaataaaaacgaa

SEQ ID NO: 189 - DNA, 25 bp, Artificial Sequence
  Synthetic
ttttcgatatcgatatcgaaggcgt

SEQ ID NO: 190 - DNA, 25 bp, Artificial Sequence
  Synthetic
ataacttaaaaccctaaattccgcc

SEQ ID NO: 191 - DNA, 26 bp, Artificial Sequence
  Synthetic
gcgggtagtaggaagattagtagcgg

SEQ ID NO: 192 - DNA, 22 bp, Artificial Sequence
  Synthetic
ccgacttccgtacgaaaccgta

SEQ ID NO: 193 - DNA, 25 bp, Artificial Sequence
  Synthetic
taatagaggtttgcgttggaatcga

SEQ ID NO: 194 - DNA, 25 bp, Artificial Sequence
  Synthetic
aacgcaccctaaacaaaaccacgac

SEQ ID NO: 195 - DNA, 26 bp, Artificial Sequence
  Synthetic
tgaagagttgttagttcgtttagcgt

SEQ ID NO: 196 - DNA, 23 bp, Artificial Sequence
  Synthetic
gccaaaaattcgattccaacgca

SEQ ID NO: 197 - DNA, 25 bp, Artificial Sequence
  Synthetic
tagtggtaggtatagttggtagcgg

SEQ ID NO: 198 - DNA, 25 bp, Artificial Sequence
  Synthetic
atcaaaactcccctcctcgaaaacg

SEQ ID NO: 199 - DNA, 19 bp, Artificial Sequence
  Synthetic
gtttttaagcggcggtcgt

SEQ ID NO: 200 - DNA, 19 bp, Artificial Sequence
  Synthetic
aaaaaaaatcccgttcgct

SEQ ID NO: 201 - DNA, 24 bp, Artificial Sequence
  Synthetic
gcgcgcgtttattagatgaagtcg

SEQ ID NO: 202 - DNA, 27 bp, Artificial Sequence
  Synthetic
aaaatcaaaaaccacaaattcaccgcc

SEQ ID NO: 203 - DNA, 25 bp, Artificial Sequence
  Synthetic
cggggagaggaggggtaggatttac

SEQ ID NO: 204 - DNA, 25 bp, Artificial Sequence
  Synthetic
caacttaaacaccacttcctccgaa

SEQ ID NO: 205 - DNA, 20 bp, Artificial Sequence
  Synthetic
tgttttttttgttcgggcgg

SEQ ID NO: 206 - DNA, 28 bp, Artificial Sequence
  Synthetic
aaataactaactcctactctcgcccgct

SEQ ID NO: 207 - DNA, 29 bp, Artificial Sequence
  Synthetic
atagttttttaattttcgcgtttcgtcga

SEQ ID NO: 208 - DNA, 24 bp, Artificial Sequence
  Synthetic
aaaaacaactccaacccacaccgc

SEQ ID NO: 209 - DNA, 25 bp, Artificial Sequence
  Synthetic
gcgggaggagtaggttaattttcga

SEQ ID NO: 210 - DNA, 25 bp, Artificial Sequence
  Synthetic
aaaaacaaaatacgcgaaacgcacg

SEQ ID NO: 211 - DNA, 26 bp, Artificial Sequence
  Synthetic
cgagaaggttttgtcgtagacgtcgt

SEQ ID NO: 212 - DNA, 22 bp, Artificial Sequence
  Synthetic
tacgtatccatacccgcgctcg

SEQ ID NO: 213 - DNA, 25 bp, Artificial Sequence
  Synthetic
tttgtttgtataataggggttgcgg

SEQ ID NO: 214 - DNA, 25 bp, Artificial Sequence
  Synthetic
cgcctaactaccgaaaaataccgaa

SEQ ID NO: 215 - DNA, 30 bp, Artificial Sequence
  Synthetic
ggtggggttatttttttatggagtcgattc

SEQ ID NO: 216 - DNA, 24 bp, Artificial Sequence
  Synthetic
cgaaccaaacctacgattcccgaa

SEQ ID NO: 217 - DNA, 27 bp, Artificial Sequence
  Synthetic
gggagaagagaatggttttttgtcgtc

SEQ ID NO: 218 - DNA, 27 bp, Artificial Sequence
  Synthetic
tcttatactcaaccccgacctaccgac

SEQ ID NO: 219 - DNA, 31 bp, Artificial Sequence
  Synthetic
gttttattcggggttttagcgttatttacgg

SEQ ID NO: 220 - DNA, 24 bp, Artificial Sequence
  Synthetic
aaaaaaccgcgttactcaacgcgc

SEQ ID NO: 221 - DNA, 24 bp, Artificial Sequence
  Synthetic
gtttagagcggaggtagcggttgc

SEQ ID NO: 222 - DNA, 26 bp, Artificial Sequence
  Synthetic
cgcctattcttaaacctaaacccgtc

SEQ ID NO: 223 - DNA, 27 bp, Artificial Sequence
  Synthetic
cgtagaggattataaagatttgtacga

SEQ ID NO: 224 - DNA, 30 bp, Artificial Sequence
  Synthetic
tactataactactacgataacgacgacgac

SEQ ID NO: 225 - DNA, 28 bp, Artificial Sequence
  Synthetic
agatttcggtttttgtttcgattttcgt

SEQ ID NO: 226 - DNA, 25 bp, Artificial Sequence
  Synthetic
attaatactaacttacgaaaccgcc

SEQ ID NO: 227 - DNA, 25 bp, Artificial Sequence
  Synthetic
attatttttgagcgtgaaaaatcgt

SEQ ID NO: 228 - DNA, 26 bp, Artificial Sequence
  Synthetic
aaatttctctccaattaaattccgta

SEQ ID NO: 229 - DNA, 22 bp, Artificial Sequence
  Synthetic
gtgggtttgtcgtcggatttcg

SEQ ID NO: 230 - DNA, 25 bp, Artificial Sequence
  Synthetic
aaataaccgcgtcatccgattcgtt

SEQ ID NO: 231 - DNA, 34 bp, Artificial Sequence
  Synthetic
tggatgttttatattaatttttagttgtataacg

SEQ ID NO: 232 - DNA, 31 bp, Artificial Sequence
  Synthetic
gtactttttctctcacgaaaaatattcccgc

SEQ ID NO: 233 - DNA, 25 bp, Artificial Sequence
  Synthetic
tgcgtggaataaattttatatacgt

SEQ ID NO: 234 - DNA, 25 bp, Artificial Sequence
  Synthetic
gctcaacacacgaaaaaccctcgaa

SEQ ID NO: 235 - DNA, 25 bp, Artificial Sequence
  Synthetic
cggtgcggggttttaataaaggatc

SEQ ID NO: 236 - DNA, 25 bp, Artificial Sequence
  Synthetic
tccacgcaaaaacaaaaaacgcgta

SEQ ID NO: 237 - DNA, 27 bp, Artificial Sequence
  Synthetic
ggcgtagttatgatttcgttttttcgt

SEQ ID NO: 238 - DNA, 26 bp, Artificial Sequence
  Synthetic
atcctttcgaccctacgtacctcgat

SEQ ID NO: 239 - DNA, 28 bp, Artificial Sequence
  Synthetic
tttacgattattgttttagataatacgg

SEQ ID NO: 240 - DNA, 19 bp, Artificial Sequence
  Synthetic
gaacccgacgaacttcgaa

SEQ ID NO: 241 - DNA, 21 bp, Artificial Sequence
  Synthetic
gggaaatcgcgtagtttgggc

SEQ ID NO: 242 - DNA, 25 bp, Artificial Sequence
  Synthetic
aaaacgacgaaaaaacgaaaacgac

SEQ ID NO: 243 - DNA, 26 bp, Artificial Sequence
  Synthetic
agttatcgcgatcggtttgggttaac

SEQ ID NO: 244 - DNA, 28 bp, Artificial Sequence
  Synthetic
aaacgattacctctttcgttcgttcgtt

SEQ ID NO: 245 - DNA, 24 bp, Artificial Sequence
  Synthetic
cggcggtttatttgaagagggttc

SEQ ID NO: 246 - DNA, 25 bp, Artificial Sequence
  Synthetic
cgacaaatcaaaaatctacaacgct

SEQ ID NO: 247 - DNA, 25 bp, Artificial Sequence
  Synthetic
ttttaacgttagttacgagttgcgg

SEQ ID NO: 248 - DNA, 21 bp, Artificial Sequence
  Synthetic
cgaacaaaccaaacaaccgaa

SEQ ID NO: 249 - DNA, 19 bp, Artificial Sequence
  Synthetic
gtagattaggcgggggcga

SEQ ID NO: 250 - DNA, 34 bp, Artificial Sequence
  Synthetic
gaacaaaaacataaactaatacaaatatctcccg

SEQ ID NO: 251 - DNA, 24 bp, Artificial Sequence
  Synthetic
ggagggagagtttttcgcggattc

SEQ ID NO: 252 - DNA, 25 bp, Artificial Sequence
  Synthetic
ctaaacccctcaaaccctaaccgat

SEQ ID NO: 253 - DNA, 20 bp, Artificial Sequence
  Synthetic
tgttttcggatacggcgagc

SEQ ID NO: 254 - DNA, 23 bp, Artificial Sequence
  Synthetic
acgaacgaactatacgcgacgct

SEQ ID NO: 255 - DNA, 21 bp, Artificial Sequence
  Synthetic
tggtaatcgggtttttcgacg

SEQ ID NO: 256 - DNA, 22 bp, Artificial Sequence
  Synthetic
ccgcgaatctatctaccgaaac

SEQ ID NO: 257 - DNA, 19 bp, Artificial Sequence
  Synthetic
gtgttaggttgggcggaag

SEQ ID NO: 258 - DNA, 22 bp, Artificial Sequence
  Synthetic
gttacccgcttacgaaaaacga

SEQ ID NO: 259 - DNA, 24 bp, Artificial Sequence
  Synthetic
ttcgttttttgtcgggagttattc

SEQ ID NO: 260 - DNA, 28 bp, Artificial Sequence
  Synthetic
tccaaaaattaaattaaaaacgctacgc

SEQ ID NO: 261 - DNA, 21 bp, Artificial Sequence
  Synthetic
ataatacggttgttcgggagg

SEQ ID NO: 262 - DNA, 25 bp, Artificial Sequence
  Synthetic
gtaaatataaactacgcgacgcgta

SEQ ID NO: 263 - DNA, 21 bp, Artificial Sequence
  Synthetic
gagagtttaggtagcgttcgg

SEQ ID NO: 264 - DNA, 28 bp, Artificial Sequence
  Synthetic
cctaacgctactaacaacattataacga

SEQ ID NO: 265 - DNA, 19 bp, Artificial Sequence
  Synthetic
cgcggttttggagcgttag

SEQ ID NO: 266 - DNA, 20 bp, Artificial Sequence
  Synthetic
ccgaaacgaccgaaaacgac

SEQ ID NO: 267 - DNA, 20 bp, Artificial Sequence
  Synthetic
cggttcgttgcgtttatcga

SEQ ID NO: 268 - DNA, 20 bp, Artificial Sequence
  Synthetic
cccccgaactactctacgcg

SEQ ID NO: 269 - DNA, 28 bp, Artificial Sequence
  Synthetic
gattatattcggattttgtttatcgcgt

SEQ ID NO: 270 - DNA, 18 bp, Artificial Sequence
  Synthetic
gactcttcctacccgcga

SEQ ID NO: 271 - DNA, 19 bp, Artificial Sequence
  Synthetic
gcggtttttagttcgcggg

SEQ ID NO: 272 - DNA, 27 bp, Artificial Sequence
  Synthetic
aacaaataattaacaaacaacgcctcc

SEQ ID NO: 273 - DNA, 24 bp, Artificial Sequence
  Synthetic
tcgttcggcgtatttatttcgtat

SEQ ID NO: 274 - DNA, 19 bp, Artificial Sequence
  Synthetic
cgcgaaaaacttcctccga

SEQ ID NO: 275 - DNA, 20 bp, Artificial Sequence
  Synthetic
ggattggtgagattcgggac

SEQ ID NO: 276 - DNA, 21 bp, Artificial Sequence
  Synthetic
cccgaaaccaaaaaacaacga

SEQ ID NO: 277 - DNA, 21 bp, Artificial Sequence
  Synthetic
cggggagtttcgtttgtatcg

SEQ ID NO: 278 - DNA, 26 bp, Artificial Sequence
  Synthetic
cgaataacgactacgaactttaaacg

SEQ ID NO: 279 - DNA, 28 bp, Artificial Sequence
  Synthetic
cgtagttatagatttattagagagggcg

SEQ ID NO: 280 - DNA, 26 bp, Artificial Sequence
  Synthetic
ctaaaacgataaaaaaacgcgaaacg

SEQ ID NO: 281 - DNA, 23 bp, Artificial Sequence
  Synthetic
tggtagttttcggtatcgacgag

SEQ ID NO: 282 - DNA, 20 bp, Artificial Sequence
  Synthetic
taactctacgcgcaaaacgc

SEQ ID NO: 283 - DNA, 20 bp, Artificial Sequence
  Synthetic
gggatttttagcggaagcga

SEQ ID NO: 284 - DNA, 23 bp, Artificial Sequence
  Synthetic
cgacgaactatccgactatcact

SEQ ID NO: 285 - DNA, 21 bp, Artificial Sequence
  Synthetic
cggaggaatcgggtagaatcg

SEQ ID NO: 286 - DNA, 22 bp, Artificial Sequence
  Synthetic
actctcccataacaacgactcc

SEQ ID NO: 287 - DNA, 17 bp, Artificial Sequence
  Synthetic
cgcgtagggcgagtttc

SEQ ID NO: 288 - DNA, 18 bp, Artificial Sequence
  Synthetic
gcctcctcctacctctcg

SEQ ID NO: 289 - DNA, 22 bp, Artificial Sequence
  Synthetic
tcggcggtttttagtaaaagcg

SEQ ID NO: 290 - DNA, 19 bp, Artificial Sequence
  Synthetic
aaatctcccgtcccactcc

SEQ ID NO: 291 - DNA, 20 bp, Artificial Sequence
  Synthetic
ggtatattcgcgtaggtgcg

SEQ ID NO: 292 - DNA, 25 bp, Artificial Sequence
  Synthetic
aaccgaataccgaaatctataaccc

SEQ ID NO: 293 - DNA, 21 bp, Artificial Sequence
  Synthetic
gtagttgggttgtagtgcgtg

SEQ ID NO: 294 - DNA, 19 bp, Artificial Sequence
  Synthetic
cccgaacttcccatcgaac

SEQ ID NO: 295 - DNA, 23 bp, Artificial Sequence
  Synthetic
ttcgtacggttttttcgttttcg

SEQ ID NO: 296 - DNA, 26 bp, Artificial Sequence
  Synthetic
ccaccacgtaataattcttctcgaaa

SEQ ID NO: 297 - DNA, 24 bp, Artificial Sequence
  Synthetic
cggtttgatattattcggggttcg

SEQ ID NO: 298 - DNA, 23 bp, Artificial Sequence
  Synthetic
aattaacgccccctataacatcc

SEQ ID NO: 299 - DNA, 25 bp, Artificial Sequence
  Synthetic
cgcgatagcgttttttattgtcgcg

SEQ ID NO: 300 - DNA, 21 bp, Artificial Sequence
  Synthetic
cgcacgaccgtaaaatactcg

SEQ ID NO: 301 - DNA, 24 bp, Artificial Sequence
  Synthetic
cggttcgtagattgttttagagcg

SEQ ID NO: 302 - DNA, 32 bp, Artificial Sequence
  Synthetic
caaataccgtcgaaaaaaaactaaatcaaaac

SEQ ID NO: 303 - DNA, 21 bp, Artificial Sequence
  Synthetic
cgttgtaggacggttatgtcg

SEQ ID NO: 304 - DNA, 25 bp, Artificial Sequence
  Synthetic
catcctactcttcgaaataaaccgc

SEQ ID NO: 305 - DNA, 26 bp, Artificial Sequence
  Synthetic
agtcgtttttttaggtagtttaggcg

SEQ ID NO: 306 - DNA, 19 bp, Artificial Sequence
  Synthetic
cgacctttacaatcgccgc

SEQ ID NO: 307 - DNA, 19 bp, Artificial Sequence
  Synthetic
agattggcgcgtaaaagcg

SEQ ID NO: 308 - DNA, 17 bp, Artificial Sequence
  Synthetic
accgaccccgaaaaacg

SEQ ID NO: 309 - DNA, 18 bp, Artificial Sequence
  Synthetic
cgttttcggagtcgcgtg

SEQ ID NO: 310 - DNA, 26 bp, Artificial Sequence
  Synthetic
aaccatacttatccgaacgtctaaac

SEQ ID NO: 311 - DNA, 21 bp, Artificial Sequence
  Synthetic
gagtagggttattttcgcggg

SEQ ID NO: 312 - DNA, 29 bp, Artificial Sequence
  Synthetic
ctacttttttcccgacaaaataaaaacgt

SEQ ID NO: 313 - DNA, 21 bp, Artificial Sequence
  Synthetic
ttttcgcgtatttcgtggttc

SEQ ID NO: 314 - DNA, 16 bp, Artificial Sequence
  Synthetic
aacgccgccgtattcg

SEQ ID NO: 315 - DNA, 17 bp, Artificial Sequence
  Synthetic
tcgcgttggaagttgcg

SEQ ID NO: 316 - DNA, 25 bp, Artificial Sequence
  Synthetic
cgtattctaaacgctaaaaaaccgc

SEQ ID NO: 317 - DNA, 17 bp, Artificial Sequence
  Synthetic
cggcggtagttttgcgg

SEQ ID NO: 318 - DNA, 25 bp, Artificial Sequence
  Synthetic
ctactaaacaaaaaccaacacgtcc

SEQ ID NO: 319 - DNA, 24 bp, Artificial Sequence
  Synthetic
ggtaggtttgttagttggttttcg

SEQ ID NO: 320 - DNA, 20 bp, Artificial Sequence
  Synthetic
cgctatctctacgaccgcct

SEQ ID NO: 321 - DNA, 17 bp, Artificial Sequence
  Synthetic
cggaggtagcgggcgag

SEQ ID NO: 322 - DNA, 17 bp, Artificial Sequence
  Synthetic
cactcaccgcttccgcc

SEQ ID NO: 323 - DNA, 16 bp, Artificial Sequence
  Synthetic
ggcgttcgtttcggcg

SEQ ID NO: 324 - DNA, 16 bp, Artificial Sequence
  Synthetic
cgcttctccgacgccc

SEQ ID NO: 325 - DNA, 20 bp, Artificial Sequence
  Synthetic
gcggttgagtttttggtcgg

SEQ ID NO: 326 - DNA, 24 bp, Artificial Sequence
  Synthetic
ccccgtataactaaaaacgacgac

SEQ ID NO: 327 - DNA, 31 bp, Artificial Sequence
  Synthetic
cgttttttttatgtagtaagcgatttttcgc

SEQ ID NO: 328 - DNA, 17 bp, Artificial Sequence
  Synthetic
aaacgacgacgaacgcc

SEQ ID NO: 329 - DNA, 24 bp, Artificial Sequence
  Synthetic
gcgttttggttttttcgtttcgag

SEQ ID NO: 330 - DNA, 21 bp, Artificial Sequence
  Synthetic
gaacgacgaaactaaaaccgc

SEQ ID NO: 331 - DNA, 27 bp, Artificial Sequence
  Synthetic
cgttttttggtagtttttttcgagtcg

SEQ ID NO: 332 - DNA, 22 bp, Artificial Sequence
  Synthetic
gcttaaacgtaaccgaaacgcc

SEQ ID NO: 333 - DNA, 19 bp, Artificial Sequence
  Synthetic
ggttgcgcgtcgttttttc

SEQ ID NO: 334 - DNA, 19 bp, Artificial Sequence
  Synthetic
cccgacgcgtttaaatcgt

SEQ ID NO: 335 - DNA, 28 bp, Artificial Sequence
  Synthetic
ggatgggaatagttaagttttagtcgtt

SEQ ID NO: 336 - DNA, 27 bp, Artificial Sequence
  Synthetic
tccaacattacatacaacactaacgtc

SEQ ID NO: 337 - DNA, 21 bp, Artificial Sequence
  Synthetic
ggttaggggtggagttcgtta

SEQ ID NO: 338 - DNA, 24 bp, Artificial Sequence
  Synthetic
actccgaactctactcatcctttc

SEQ ID NO: 339 - DNA, 21 bp, Artificial Sequence
  Synthetic
taggttggagattttgacgcg

SEQ ID NO: 340 - DNA, 22 bp, Artificial Sequence
  Synthetic
cgaaacctaaaaacgccgaaac

SEQ ID NO: 341 - DNA, 25 bp, Artificial Sequence
  Synthetic
ggttggtagtcgtttttacgttttc

SEQ ID NO: 342 - DNA, 30 bp, Artificial Sequence
  Synthetic
caaaacccatctaattacaaaatacctcga

SEQ ID NO: 343 - DNA, 19 bp, Artificial Sequence
  Synthetic
tggagttatcggaaggcga

SEQ ID NO: 344 - DNA, 18 bp, Artificial Sequence
  Synthetic
cgaactcccgaaacgacg

SEQ ID NO: 345 - DNA, 27 bp, Artificial Sequence
  Synthetic
ggaaatggtttagagttttggatttcg

SEQ ID NO: 346 - DNA, 27 bp, Artificial Sequence
  Synthetic
ttctaaaaaatactttcgataccgaca

SEQ ID NO: 347 - DNA, 29 bp, Artificial Sequence
  Synthetic
gtggtttgaagagttgttagttcgtttag

SEQ ID NO: 348 - DNA, 23 bp, Artificial Sequence
  Synthetic
gccaaaaattcgattccaacgca

SEQ ID NO: 349 - DNA, 22 bp, Artificial Sequence
  Synthetic
aaggtgggttgtttgaagaagc

SEQ ID NO: 350 - DNA, 22 bp, Artificial Sequence
  Synthetic
accctccgacaaaaaaacgtac

SEQ ID NO: 351 - DNA, 21 bp, Artificial Sequence
  Synthetic
gcgagaaggttttgtcgtaga

SEQ ID NO: 352 - DNA, 19 bp, Artificial Sequence
  Synthetic
acctactcacgcacaacct

SEQ ID NO: 353 - DNA, 17 bp, Artificial Sequence
  Synthetic
cgcggtgaggaagatcg

SEQ ID NO: 354 - DNA, 18 bp, Artificial Sequence
  Synthetic
acgccacctacgactacg

SEQ ID NO: 355 - DNA, 21 bp, Artificial Sequence
  Synthetic
gtacggttattggttgagcgg

SEQ ID NO: 356 - DNA, 19 bp, Artificial Sequence
  Synthetic
ccgaatcctcctccaaacg

SEQ ID NO: 357 - DNA, 28 bp, Artificial Sequence
  Synthetic
ggaatttaattggagagaaattttggcg

SEQ ID NO: 358 - DNA, 27 bp, Artificial Sequence
  Synthetic
ccaaaatttccctcatctatatacgcc

SEQ ID NO: 359 - DNA, 17 bp, Artificial Sequence
  Synthetic
gttgcgggtcgggttgc

SEQ ID NO: 360 - DNA, 26 bp, Artificial Sequence
  Synthetic
gcaaaaacaaaaaacgcgtaaaaacc

SEQ ID NO: 361 - DNA, 21 bp, Artificial Sequence
  Synthetic
gtcgtcgttgtcgtagttgtc

SEQ ID NO: 362 - DNA, 20 bp, Artificial Sequence
  Synthetic
cgtaaaaaccgaacgacgcg

SEQ ID NO: 363 - DNA, 26 bp, Artificial Sequence
  Synthetic
ttttcgttgattttattcgagtcgtc

SEQ ID NO: 364 - DNA, 22 bp, Artificial Sequence
  Synthetic
gaaccctcttcaaataaaccgc

SEQ ID NO: 365 - DNA, 21 bp, Artificial Sequence
  Synthetic
gattaaatagtcggggtcgcg

SEQ ID NO: 366 - DNA, 19 bp, Artificial Sequence
  Synthetic
attctccaacgccaaccac

SEQ ID NO: 367 - DNA, 24 bp, Artificial Sequence
  Synthetic
cgcgccgaggcgcgcttccactcc

SEQ ID NO: 368 - DNA, 33 bp, Artificial Sequence
  Synthetic
aggccacggacggcggcgtttttttttatgttg

SEQ ID NO: 369 - DNA, 39 bp, Artificial Sequence
  Synthetic
aggccacggacgcaaccgaactaaaaaaaaaaactaacg

SEQ ID NO: 370 - DNA, 27 bp, Artificial Sequence
  Synthetic
cgcgccgagggcgcgtaagattttcgg

SEQ ID NO: 371 - DNA, 25 bp, Artificial Sequence
  Synthetic
cgcgccgagggcgggtagtagtgcg

SEQ ID NO: 372 - DNA, 31 bp, Artificial Sequence
  Synthetic
cgcgccgaggcgaccgaaaaatcgaaaaaca

SEQ ID NO: 373 - DNA, 30 bp, Artificial Sequence
  Synthetic
cgcgccgagggctaacgcgaataaaacacg

SEQ ID NO: 374 - DNA, 29 bp, Artificial Sequence
  Synthetic
cgcgccgaggttttcgttttcggtttcgg

SEQ ID NO: 375 - DNA, 28 bp, Artificial Sequence
  Synthetic
cgcgccgaggccgtacctattaactccg

SEQ ID NO: 376 - DNA, 31 bp, Artificial Sequence
  Synthetic
aggccacggacgtcgttttttttttgcgggt

SEQ ID NO: 377 - DNA, 30 bp, Artificial Sequence
  Synthetic
aggccacggacgcgtattggcgcgatttag

SEQ ID NO: 378 - DNA, 33 bp, Artificial Sequence
  Synthetic
aggccacggacggttcgaaaaaaactcgacgaa

SEQ ID NO: 379 - DNA, 30 bp, Artificial Sequence
  Synthetic
aggccacggacggccgttctctaacttccg

SEQ ID NO: 380 - DNA, 29 bp, Artificial Sequence
  Synthetic
aggccacggacgccgaaatacgaacgcga

SEQ ID NO: 381 - DNA, 29 bp, Artificial Sequence
  Synthetic
aggccacggacgtcgttcctcgatttcgc

SEQ ID NO: 382 - DNA, 37 bp, Artificial Sequence
  Synthetic
aggccacggacgcgaataaaacctacgaaaaaaaacg

SEQ ID NO: 383 - DNA, 31 bp, Artificial Sequence
  Synthetic
aggccacggacggaaaaccgcaaaatcctcg

SEQ ID NO: 384 - DNA, 38 bp, Artificial Sequence
  Synthetic
aggccacggacgcgcgaaataaacctataattaactca

SEQ ID NO: 385 - DNA, 29 bp, Artificial Sequence
  Synthetic
cgcgccgaggccgaaccaacactcaaaac

SEQ ID NO: 386 - DNA, 26 bp, Artificial Sequence
  Synthetic
cgcgccgagggcgcgtttggtttggt

SEQ ID NO: 387 - DNA, 26 bp, Artificial Sequence
  Synthetic
aggccacggacgaacgcgctccaacc

SEQ ID NO: 388 - DNA, 31 bp, Artificial Sequence
  Synthetic
cgcgccgaggcgcgacgactaaaaaaattca

SEQ ID NO: 389 - DNA, 30 bp, Artificial Sequence
  Synthetic
aggccacggacggtcgaaatcgaaacgctc

SEQ ID NO: 390 - DNA, 26 bp, Artificial Sequence
  Synthetic
cgcgccgaggccgcgactacctcttc

SEQ ID NO: 391 - DNA, 30 bp, Artificial Sequence
  Synthetic
aggccacggacgcgacgtcctacaaaacca

SEQ ID NO: 392 - DNA, 25 bp, Artificial Sequence
  Synthetic
cgcgccgaggggcggtagttgttgc

SEQ ID NO: 393 - DNA, 24 bp, Artificial Sequence
  Synthetic
cgcgccgagggcgaaaaccccgcc

SEQ ID NO: 394 - DNA, 32 bp, Artificial Sequence
  Synthetic
cgcgccgaggcgtctaactaaacgcgataaac

SEQ ID NO: 395 - DNA, 29 bp, Artificial Sequence
  Synthetic
cgcgccgagggcggttttagcgatgaatc

SEQ ID NO: 396 - DNA, 24 bp, Artificial Sequence
  Synthetic
cgcgccgaggcgattcgagggcgt

SEQ ID NO: 397 - DNA, 27 bp, Artificial Sequence
  Synthetic
aggccacggacgcgcgacgcaaaactc

SEQ ID NO: 398 - DNA, 26 bp, Artificial Sequence
  Synthetic
aggccacggacggcggcggttggatt

SEQ ID NO: 399 - DNA, 31 bp, Artificial Sequence
  Synthetic
aggccacggacgtcccgaaacgaacgataaa

SEQ ID NO: 400 - DNA, 24 bp, Artificial Sequence
  Synthetic
cgcgccgaggcgccgtcgcactac

SEQ ID NO: 401 - DNA, 26 bp, Artificial Sequence
  Synthetic
aggccacggacgcgcgactccccact

SEQ ID NO: 402 - DNA, 32 bp, Artificial Sequence
  Synthetic
aggccacggacgcgcaaataataacgcgaacg

SEQ ID NO: 403 - DNA, 33 bp, Artificial Sequence
  Synthetic
aggccacggacgcgttcgaggttagttttttgg

SEQ ID NO: 404 - DNA, 27 bp, Artificial Sequence
  Synthetic
aggccacggacgcgtacgtaacccgcg

SEQ ID NO: 405 - DNA, 29 bp, Artificial Sequence
  Synthetic
cgcgccgaggcgctactaaccataaccgc

SEQ ID NO: 406 - DNA, 30 bp, Artificial Sequence
  Synthetic
cgcgccgaggcgttttcgtttgattcggtt

SEQ ID NO: 407 - DNA, 29 bp, Artificial Sequence
  Synthetic
cgcgccgaggtcggtgattgatgtgtgcg

SEQ ID NO: 408 - DNA, 31 bp, Artificial Sequence
  Synthetic
cgcgccgaggcgtaactccatctcgataacc

SEQ ID NO: 409 - DNA, 26 bp, Artificial Sequence
  Synthetic
cgcgccgaggcgaccgcgaaaaaacg

SEQ ID NO: 410 - DNA, 28 bp, Artificial Sequence
  Synthetic
aggccacggacgcgcgttggaagtttcg

SEQ ID NO: 411 - DNA, 26 bp, Artificial Sequence
  Synthetic
cgcgccgagggcgcgaacacaaaacg

SEQ ID NO: 412 - DNA, 27 bp, Artificial Sequence
  Synthetic
cgcgccgaggaccgaaaacgccctaaa

SEQ ID NO: 413 - DNA, 31 bp, Artificial Sequence
  Synthetic
cgcgccgagggcgtggagaaatgttagtttg

SEQ ID NO: 414 - DNA, 28 bp, Artificial Sequence
  Synthetic
aggccacggacgcgggcggtgaatttgt

SEQ ID NO: 415 - DNA, 29 bp, Artificial Sequence
  Synthetic
aggccacggacgacgtcgtatttgtggcg

SEQ ID NO: 416 - DNA, 27 bp, Artificial Sequence
  Synthetic
aggccacggacggcgttgtttagcgcg

SEQ ID NO: 417 - DNA, 30 bp, Artificial Sequence
  Synthetic
aggccacggacggatcccgcaaatcaacac

SEQ ID NO: 418 - DNA, 25 bp, Artificial Sequence
  Synthetic
cgcgccgaggcgatccccaactccc

SEQ ID NO: 419 - DNA, 30 bp, Artificial Sequence
  Synthetic
cgcgccgaggcgcttctaaaacctcgatcc

SEQ ID NO: 420 - DNA, 31 bp, Artificial Sequence
  Synthetic
cgcgccgaggcgcggtcgttaatatgtattc

SEQ ID NO: 421 - DNA, 32 bp, Artificial Sequence
  Synthetic
aggccacggacgcgtttggcgtagatataagc

SEQ ID NO: 422 - DNA, 32 bp, Artificial Sequence
  Synthetic
aggccacggacgcgaactacgaaaacaacctc

SEQ ID NO: 423 - DNA, 20 bp, Artificial Sequence
  Synthetic
ggattggtgagattcgggac

SEQ ID NO: 424 - DNA, 21 bp, Artificial Sequence
  Synthetic
cccgaaaccaaaaaacaacga

SEQ ID NO: 425 - DNA, 21 bp, Artificial Sequence
  Synthetic
gagtagggttattttcgcggg

SEQ ID NO: 426 - DNA, 29 bp, Artificial Sequence
  Synthetic
ctacttttttcccgacaaaataaaaacgt

SEQ ID NO: 427 - DNA, 25 bp, Artificial Sequence
  Synthetic
cgcgatagcgttttttattgtcgcg

SEQ ID NO: 428 - DNA, 21 bp, Artificial Sequence
  Synthetic
cgcacgaccgtaaaatactcg

SEQ ID NO: 429 - DNA, 20 bp, Artificial Sequence
  Synthetic
cggttcgttgcgtttatcga

SEQ ID NO: 430 - DNA, 20 bp, Artificial Sequence
  Synthetic
cccccgaactactctacgcg

SEQ ID NO: 431 - DNA, 21 bp, Artificial Sequence
  Synthetic
gattaaatagtcggggtcgcg

SEQ ID NO: 432 - DNA, 19 bp, Artificial Sequence
  Synthetic
attctccaacgccaaccac

SEQ ID NO: 433 - DNA, 21 bp, Artificial Sequence
  Synthetic
gtacggttattggttgagcgg

SEQ ID NO: 434 - DNA, 19 bp, Artificial Sequence
  Synthetic
ccgaatcctcctccaaacg

SEQ ID NO: 435-436 - skipped (2 entries)

SEQ ID NO: 437 - DNA, 20 bp, Artificial Sequence
  Synthetic
gggatttttagcggaagcga

SEQ ID NO: 438 - DNA, 23 bp, Artificial Sequence
  Synthetic
cgacgaactatccgactatcact

SEQ ID NO: 439 - DNA, 21 bp, Artificial Sequence
  Synthetic
ggttaggggtggagttcgtta

SEQ ID NO: 440 - DNA, 24 bp, Artificial Sequence
  Synthetic
actccgaactctactcatcctttc

SEQ ID NO: 441 - DNA, 22 bp, Artificial Sequence
  Synthetic
tcggcggtttttagtaaaagcg

SEQ ID NO: 442 - DNA, 19 bp, Artificial Sequence
  Synthetic
aaatctcccgtcccactcc

SEQ ID NO: 443 - DNA, 25 bp, Artificial Sequence
  Synthetic
ggttggtagtcgtttttacgttttc

SEQ ID NO: 444 - DNA, 30 bp, Artificial Sequence; identical to SEQ ID NO: 342
  Synthetic

SEQ ID NO: 445 - DNA, 19 bp, Artificial Sequence
  Synthetic
tggagttatcggaaggcga

SEQ ID NO: 446 - DNA, 18 bp, Artificial Sequence
  Synthetic
cgaactcccgaaacgacg

SEQ ID NO: 447 - DNA, 26 bp, Artificial Sequence
  Synthetic
ttttcgttgattttattcgagtcgtc

SEQ ID NO: 448 - DNA, 22 bp, Artificial Sequence
  Synthetic
gaaccctcttcaaataaaccgc

SEQ ID NO: 449 - DNA, 28 bp, Artificial Sequence
  Synthetic
gattatattcggattttgtttatcgcgt

SEQ ID NO: 450 - DNA, 18 bp, Artificial Sequence
  Synthetic
gactcttcctacccgcga

SEQ ID NO: 451 - DNA, 30 bp, Artificial Sequence; identical to SEQ ID NO: 377
  Synthetic

SEQ ID NO: 452 - DNA, 29 bp, Artificial Sequence
  Synthetic
cgcgccgagggcggttttagcgatgaatc

SEQ ID NO: 453 - DNA, 30 bp, Artificial Sequence; identical to SEQ ID NO: 389
  Synthetic

SEQ ID NO: 454 - DNA, 30 bp, Artificial Sequence; identical to SEQ ID NO: 373
  Synthetic

SEQ ID NO: 455 - DNA, 32 bp, Artificial Sequence; identical to SEQ ID NO: 422
  Synthetic

SEQ ID NO: 456 - DNA, 30 bp, Artificial Sequence; identical to SEQ ID NO: 417
  Synthetic

SEQ ID NO: 457 - skipped

SEQ ID NO: 458 - DNA, 27 bp, Artificial Sequence
  Synthetic
cgcgccgaggtcgttcctcgatttcgc

SEQ ID NO: 459 - DNA, 31 bp, Artificial Sequence; identical to SEQ ID NO: 408
  Synthetic

SEQ ID NO: 460 - DNA, 36 bp, Artificial Sequence
  Synthetic
cgcgccgaggcgcgaaataaacctataattaactca

SEQ ID NO: 461 - DNA, 28 bp, Artificial Sequence
  Synthetic
aggccacggacgcgcgttggaagtttcg

SEQ ID NO: 462 - DNA, 26 bp, Artificial Sequence
  Synthetic
cgcgccgagggcgcgaacacaaaacg

SEQ ID NO: 463 - DNA, 32 bp, Artificial Sequence; identical to SEQ ID NO: 421
  Synthetic

SEQ ID NO: 464 - DNA, 29 bp, Artificial Sequence
  Synthetic
cgcgccgaggttttcgttttcggtttcgg